European Patent Application EP 4 552 649 A2, published May 14, 2025. Title: THERAPY GUIDANCE AND/OR THERAPY MONITORING FOR TREATMENT OF SHOCK. Applicant: 4Teen4 Pharmaceuticals GmbH. Application EP. The sequence listing filed with the application follows.

SEQUENCE LISTING (61 sequences)

SEQ ID NO: 1 - protein, 737 aa, Homo sapiens
MADTQYILPNDIGVSSLDCREAFRLLSPTERLYAYHLSRAAWYGGLAVLLQTSPEAPYIYALLSRLFRAQDPDQLRQHALAEGLTEEEYQAFLVYAAGVYSNMGNYKSFGDTKFVPNLPKEKLERVILGSEAAQQHPEEVRGLWQTCGELMFSLEPRLRHLGLGKEGITTYFSGNCTMEDAKLAQDFLDSQNLSAYNTRLFKEVDGEGKPYYEVRLASVLGSEPSLDSEVTSKLKSYEFRGSPFQVTRGDYAPILQKVVEQLEKAKAYAANSHQGQMLAQYIESFTQGSIEAHKRGSRFWIQDKGPIVESYIGFIESYRDPFGSRGEFEGFVAVVNKAMSAKFERLVASAEQLLKELPWPPTFEKDKFLTPDFTSLDVLTFAGSGIPAGINIPNYDDLRQTEGFKNVSLGNVLAVAYATQREKLTFLEEDDKDLYILWKGPSFDVQVGLHELLGHGSGKLFVQDEKGAFNFDQETVINPETGEQIQSWYRSGETWDSKFSTIASSYEECRAESVGLYLCLHPQVLEIFGFEGADAEDVIYVNWLNMVRAGLLALEFYTPEAFNWRQAHMQARFVILRVLLEAGEGLVTITPTTGSDGRPDARVRLDRSKIRSVGKPALERFLRRLQVLKSTGDVAGGRALYEGYATVTDAPPECFLTLRDTVLLRKESRKLIVQPNTRLEGSDVQLLEYEASAAGLIRSFSERFPEDGPELEEILTQLATADARFWKGPSEAPSGQA

SEQ ID NO: 2 - protein, 21 aa, Synthetic construct
CETVINPETGEQIQSWYRSGE

SEQ ID NO: 3 - protein, 6 aa, Homo sapiens
INPETG

SEQ ID NO: 4 - protein, 116 aa, Synthetic construct
QVTLKESGPGILQPSQTLSLTCSFSGFSLSTSGMSVGWIRQPSGKGLEWLAHIWWNDNKSYNPALKSRLTISRDTSNNQVFLKIASVVTADTGTYFCARNYSYDYWGQGTTLTVSS

SEQ ID NO: 5 - protein, 112 aa, Synthetic construct
DVVVTQTPLSLSVSLGDPASISCRSSRSLVHSIGSTYLHWYLQKPGQSPKLLIYKVSNRFSGVPDRFSGSGSGTDFTLKISRVEAEDLGVYFCSQSTHVPWTFGGGTKLEIK

SEQ ID NO: 6 - protein, 10 aa, Synthetic construct
GFSLSTSGMS

SEQ ID NO: 7 - protein, 7 aa, Synthetic construct
IWWNDNK

SEQ ID NO: 8 - protein, 8 aa, Synthetic construct
ARNYSYDY

SEQ ID NO: 9 - protein, 11 aa, Synthetic construct
RSLVHSIGSTY

SEQ ID NO: 10 - protein, 9 aa, Synthetic construct
SQSTHVPWT

SEQ ID NO: 11 - protein, 469 aa, Synthetic construct
MDPKGSLSWRILLFLSLAFELSYGQITLKESGPTLVKPTQTLTLTCTFSGFSLSTSGMSVGWIRQPPGKALEWLAHIWWNDNKSYNPALKSRLTITRDTSKNQVVLTMTNMDPVDTGTYYCARNYSYDYWGQGTLVTVSSASTKGPSVFPLAPSSKSTSGGTAALGCLVKDYFPEPVTVSWNSGALTSGVHTFPAVLQSSGLYSLSSVVTVPSSSLGTQTYICNVNHKPSNTKVDKKVEPKSCDKTHTCPPCPAPELLGGPSVFLFPPKPKDTLMISRTPEVTCVVVDVSHEDPEVKFNWYVDGVEVHNAKTKPREEQYNSTYRVVSVLTVLHQDWLNGKEYKCKVSNKALPAPIEKTISKAKGQPREPQVYTLPPSRDELTKNQVSLTCLVKGFYPSDIAVEWESNGQPENNYKTTPPVLDSDGSFFLYSKLTVDKSRWQQGNVFSCSVMHEALHNHYTQKSLSLSPG

SEQ ID NO: 12 - protein, 239 aa, Synthetic construct
METDTLLLWVLLLWVPGSTGDIVMTQTPLSLSVTPGQPASISCKSSRSLVHSIGSTYLYWYLQKPGQSPQLLIYKVSNRFSGVPDRFSGSGSGTDFTLKISRVEAEDVGVYYCSQSTHVPWTFGGGTKVEIKRTVAAPSVFIFPPSDEQLKSGTASVVCLLNNFYPREAKVQWKVDNALQSGNSQESVTEQDSKDSTYSLSSTLTLSKADYEKHKVYACEVTHQGLSSPVTKSFNRGEC

SEQ ID NO: 13 - protein, 8 aa, Homo sapiens
DRVYIHPF

SEQ ID NO: 14 - protein, 8 aa, Synthetic construct
DRVYVHPF

SEQ ID NO: 15 - protein, 8 aa, Synthetic construct
NRVFIHPF

SEQ ID NO: 16 - protein, 6 aa, Synthetic construct
VYIHPF

SEQ ID NO: 17 - protein, 9 aa, Synthetic construct
NRVYYVHPF

SEQ ID NO: 18 - protein, 8 aa, Synthetic construct
NRVYIHPI

SEQ ID NO: 19 - protein, 8 aa, Synthetic construct
NRVYIHPA

SEQ ID NO: 20 - protein, 8 aa, Synthetic construct
  MOD_RES 4: note = Diiodo-Tyrosine
NRVYIHPF

SEQ ID NO: 21 - protein, 7 aa, Homo sapiens
RVYIHPF

SEQ ID NO: 22 - protein, 7 aa, Synthetic construct
RVYVHPF

SEQ ID NO: 23 - protein, 7 aa, Synthetic construct
RVFIHPF

SEQ ID NO: 24 - protein, 7 aa, Synthetic construct
RVYIHPA

SEQ ID NO: 25 - protein, 7 aa, Synthetic construct
  MOD_RES 3: note = Diiodo-Tyrosine
RVYIHPF

SEQ ID NO: 26 - protein, 6 aa, Homo sapiens
VYIHPF

SEQ ID NO: 27 - protein, 6 aa, Synthetic construct
VYVHPF

SEQ ID NO: 28 - protein, 6 aa, Synthetic construct
VFIHPF

SEQ ID NO: 29 - protein, 6 aa, Synthetic construct
VYIHPA

SEQ ID NO: 30 - protein, 6 aa, Synthetic construct
  MOD_RES 2: note = Diiodo-Tyrosine
VYIHPF

SEQ ID NO: 31 - protein, 164 aa, Homo sapiens
ARLDVASEFRKKWNKWALSRGKRELRMSSSYPTGLADVKAGPAQTLIRPQDMKGASRSPEDSSPDAARIRVKRYRQSMNNFQGLRSFGCRFGTCTVQKLAHQIYQFTDKDKDNVAPRSKISPQGYGRRRRRSLPEAGPGRTLVSSKPQAHGAPAPPSGSAPHFL

SEQ ID NO: 32 - protein, 20 aa, Homo sapiens
ARLDVASEFRKKWNKWALSR

SEQ ID NO: 33 - protein, 48 aa, Homo sapiens
ELRMSSSYPTGLADVKAGPAQTLIRPQDMKGASRSPEDSSPDAARIRV

SEQ ID NO: 34 - protein, 52 aa, Homo sapiens
  MOD_RES 52: note = C-terminal amidation
YRQSMNNFQGLRSFGCRFGTCTVQKLAHQIYQFTDKDKDNVAPRSKISPQGY

SEQ ID NO: 35 - protein, 53 aa, Homo sapiens
YRQSMNNFQGLRSFGCRFGTCTVQKLAHQIYQFTDKDKDNVAPRSKISPQGYG

SEQ ID NO: 36 - protein, 38 aa, Homo sapiens
RRRRRSLPEAGPGRTLVSSKPQAHGAPAPPSGSAPHFL

SEQ ID NO: 37 - protein, 21 aa, Homo sapiens
YRQSMNNFQGLRSFGCRFGTC

SEQ ID NO: 38 - protein, 8 aa, Synthetic construct
GYTFSRYW

SEQ ID NO: 39 - protein, 8 aa, Synthetic construct
ILPGSGST

SEQ ID NO: 40 - protein, 11 aa, Synthetic construct
TEGYEYDGFDY

SEQ ID NO: 41 - protein, 11 aa, Synthetic construct
QSIVYSNGNTY

SEQ ID NO: 42 - protein, 9 aa, Synthetic construct
FQGSHIPYT

SEQ ID NO: 43 - protein, 448 aa, Synthetic construct
QVQLVQSGAEVKKPGSSVKVSCKASGYTFSRYWIEWVRQAPGQGLEWIGEILPGSGSTNYNQKFQGRVTITADTSTSTAYMELSSLRSEDTAVYYCTEGYEYDGFDYWGQGTTVTVSSASTKGPSVFPLAPSSKSTSGGTAALGCLVKDYFPEPVTVSWNSGALTSGVHTFPAVLQSSGLYSLSSVVTVPSSSLGTQTYICNVNHKPSNTKVDKKVEPKSCDKTHTCPPCPAPELLGGPSVFLFPPKPKDTLMISRTPEVTCVVVDVSHEDPEVKFNWYVDGVEVHNAKTKPREEQYNSTYRVVSVLTVLHQDWLNGKEYKCKVSNKALPAPIEKTISKAKGQPREPQVYTLPPSRDELTKNQVSLTCLVKGFYPSDIAVEWESNGQPENNYKTTPPVLDSDGSFFLYSKLTVDKSRWQQGNVFSCSVMHEALHNHYTQKSLSLSPGK

SEQ ID NO: 44 - protein, 218 aa, Synthetic construct
DVVLTQSPLSLPVTLGQPASISCRSSQSIVYSNGNTYLEWYLQRPGQSPRLLIYRVSNRFSGVPDRFSGSGSGTDFTLKISRVEAEDVGVYYCFQGSHIPYTFGGGTKLEIKRTVAAPSVFIFPPSDEQLKSGTASVVCLLNNFYPREAKVQWKVDNALQSGNSQESVTEQDSKDSTYSLSSTLTLSKADYEKHKVYACEVTHQGLSSPVTKSFNRGE

SEQ ID NO: 45 - protein, 25 aa, Synthetic construct
  MOD_RES 1: note = N-terminal biotinylation
AFNFDQETVINPETGEQIQSWYRSG

SEQ ID NO: 46 - protein, 19 aa, Synthetic construct
  MOD_RES 1: note = N-terminal biotinylation
AFNFDQETVINPETGEQIQ

SEQ ID NO: 47 - protein, 18 aa, Synthetic construct
  MOD_RES 1: note = N-terminal biotinylation
AFNFDQETVINPETGEQI

SEQ ID NO: 48 - protein, 17 aa, Synthetic construct
  MOD_RES 1: note = N-terminal biotinylation
AFNFDQETVINPETGEQ

SEQ ID NO: 49 - protein, 16 aa, Synthetic construct
  MOD_RES 1: note = N-terminal biotinylation
AFNFDQETVINPETGE

SEQ ID NO: 50 - protein, 15 aa, Synthetic construct
  MOD_RES 1: note = N-terminal biotinylation
AFNFDQETVINPETG

SEQ ID NO: 51 - protein, 14 aa, Synthetic construct
  MOD_RES 1: note = N-terminal biotinylation
AFNFDQETVINPET

SEQ ID NO: 52 - protein, 13 aa, Synthetic construct
  MOD_RES 1: note = N-terminal biotinylation
AFNFDQETVINPE

SEQ ID NO: 53 - protein, 12 aa, Synthetic construct
  MOD_RES 1: note = N-terminal biotinylation
AFNFDQETVINP

SEQ ID NO: 54 - protein, 11 aa, Synthetic construct
  MOD_RES 1: note = N-terminal biotinylation
AFNFDQETVIN

SEQ ID NO: 55 - protein, 11 aa, Synthetic construct
  MOD_RES 11: note = C-terminal biotinylation
ETGEQIQSWYK

SEQ ID NO: 56 - protein, 12 aa, Synthetic construct
  MOD_RES 12: note = C-terminal biotinylation
PETGEQIQSWYK

SEQ ID NO: 57 - protein, 13 aa, Synthetic construct
  MOD_RES 13: note = C-terminal biotinylation
NPETGEQIQSWYK

SEQ ID NO: 58 - protein, 14 aa, Synthetic construct
  MOD_RES 14: note = C-terminal biotinylation
INPETGEQIQSWYK

SEQ ID NO: 59 - protein, 15 aa, Synthetic construct
  MOD_RES 15: note = C-terminal biotinylation
VINPETGEQIQSWYK

SEQ ID NO: 60 - protein, 16 aa, Synthetic construct
  MOD_RES 16: note = C-terminal biotinylation
TVINPETGEQIQSWYK

SEQ ID NO: 61 - protein, 17 aa, Synthetic construct
  MOD_RES 17: note = C-terminal biotinylation
ETVINPETGEQIQSWYK